European Patent Specification EP 4 081 244 B1, published November 26, 2025. Title: STAPLED OLEFIN CO-AGONISTS OF THE GLUCAGON AND GLP-1 RECEPTORS. Applicant: Bianchi, Elisabetta Deng, Qiaolin Lin, Songnian Orvieto, Frederica Palani, Anandan Pessi, Antonello Sawyer, Tomi. The sequence listing filed with the application follows.

SEQUENCE LISTING (20 sequences)

SEQ ID NO: 1 - protein, 29 aa, Homo sapiens
HSQGTFTSDYSKYLDSRRAQDFVQWLMNT

SEQ ID NO: 2 - protein, 30 aa, Homo sapiens
HAEGTFTSDVSSYLEGQAAKEFIAWLVKGR

SEQ ID NO: 3 - protein, 37 aa, Homo sapiens
HSQGTFTSDYSKYLDSRRAQDFVQWLMNTKRNRNNIA

SEQ ID NO: 4 - protein, 39 aa, Heloderma suspectum
HGEGTFTSDLSKQMEEEAVRLFIEWLKNGGPSSGAPPPS

SEQ ID NO: 5 - protein, 33 aa, Homo sapiens
HADGSFSDEMNTILDNLAARDFINWLIQTKITD

SEQ ID NO: 6 - protein, 29 aa, Artificial Sequence
  Peptide
  MISC_FEATURE (12)..(19): Miscellaneous feature: the alkene chain of the amino acid at position 12 forms a double bond containing ring with the alkene chain of the amino acid at position 19
  MISC_FEATURE (2)..(2): Xaa is D-Serine
  MISC_FEATURE (12)..(12): Xaa is (R)-2-amino-2-methyloct-7-enoic acid
  MISC_FEATURE (19)..(19): Xaa is (S)-2-amino-2-methylnon-8-enoic acid
  MISC_FEATURE (29)..(29): amino acid has C terminal amide
HXQGTFTSDKSXYLDERAXQDFVQWLLDT

SEQ ID NO: 7 - protein, 29 aa, Artificial Sequence
  Peptide
  MISC_FEATURE (12)..(19): Miscellaneous feature: the alkene chain of the amino acid at position 12 forms a double bond containing ring with the alkene chain of the amino acid at position 19
  MISC_FEATURE (2)..(2): Xaa is D-Serine
  MISC_FEATURE (10)..(10): Xaa is Lysine conjugated to gamma-Glu-gamma-Glu- C16 fatty acid
  MISC_FEATURE (12)..(12): Xaa is (R)-2-amino-2-methyloct-7-enoic acid
  MISC_FEATURE (19)..(19): Xaa is (S)-2-amino-2-methylnon-8-enoic acid
  MISC_FEATURE (29)..(29): amino acid has C terminal amide
HXQGTFTSDXSXYLDERAXQDFVQWLLDT

SEQ ID NO: 8 - protein, 29 aa, Artificial Sequence
  Peptide
  MISC_FEATURE (17)..(24): Miscellaneous feature: the alkene chain of the amino acid at position 17 forms a double bond containing ring with the alkene chain of the amino acid at position 24
  MISC_FEATURE (2)..(2): Xaa is D-Serine
  MISC_FEATURE (10)..(10): Xaa is Lys conjugated to gamma-Glu-gamma-Glu- C16 fatty acid
  MISC_FEATURE (17)..(17): Xaa is (R)-2-amino-2-methyloct-7-enoic acid
  MISC_FEATURE (24)..(24): Xaa is (S)-2-amino-2-methylnon-8-enoic acid
  MISC_FEATURE (29)..(29): amino acid has C terminal amide
HXQGTFTSDXSKYLDEXAAQDFVXWLLDT

SEQ ID NO: 9 - protein, 29 aa, Artificial Sequence
  Peptide
  MISC_FEATURE (17)..(24): Miscellaneous feature: the alkene chain of the amino acid at position 17 forms a double bond containing ring with the alkene chain of the amino acid at position 24
  MISC_FEATURE (2)..(2): Xaa is D-Serine
  MISC_FEATURE (17)..(17): Xaa is (R)-2-amino-2-methyloct-7-enoic acid
  MISC_FEATURE (24)..(24): Xaa is (S)-2-amino-2-methylnon-8-enoic acid
  MISC_FEATURE (29)..(29): amino acid has C terminal amide
HXQGTFTSDKSKYLDEXAAQDFVXWLLDT

SEQ ID NO: 10 - protein, 29 aa, Artificial Sequence
  Peptide
  MISC_FEATURE (20)..(27): Miscellaneous feature: the alkene chain of the amino acid at position 20 forms a double bond containing ring with the alkene chain of the amino acid at position 27
  MISC_FEATURE (2)..(2): Xaa is D-Serine
  MISC_FEATURE (10)..(10): Xaa is Lysine conjugated to gamma-Glu-gamma-Glu- C16 fatty acid
  MISC_FEATURE (20)..(20): Xaa is (R)-2-amino-2-methyloct-7-enoic acid
  MISC_FEATURE (27)..(27): Xaa is (S)-2-amino-2-methylnon-8-enoic acid
  MISC_FEATURE (29)..(29): amino acid has C terminal amide
HXQGTFTSDXSKYLDERAAXDFVQWLXDT

SEQ ID NO: 11 - protein, 29 aa, Artificial Sequence
  Peptide
  MISC_FEATURE (20)..(27): Miscellaneous feature :the alkene chain of the amino acid at position 20 forms a double bond containing ring with the alkene chain of the amino acid at position 27
  MISC_FEATURE (2)..(2): Xaa is D-Serine
  MISC_FEATURE (20)..(20): Xaa is (R)-2-amino-2-methyloct-7-enoic acid
  MISC_FEATURE (27)..(27): Xaa is (S)-2-amino-2-methylnon-8-enoic acid
  MISC_FEATURE (29)..(29): amino acid has C terminal amide
HXQGTFTSDKSKYLDERAAXDFVQWLXDT

SEQ ID NO: 12 - protein, 29 aa, Artificial Sequence
  Peptide
  MISC_FEATURE (20)..(24): Miscellaneous feature: the alkene chain of the amino acid at position 20 forms a double bond containing ring with the alkene chain of the amino acid at position 24
  MISC_FEATURE (2)..(2): Xaa is D-Serine
  MISC_FEATURE (10)..(10): Xaa is Lysine conjugated to gamma-Glu-gamma-Glu- C16 fatty acid
  MISC_FEATURE (20)..(20): Xaa is (S)-2-amino-2-methylhept-6-enoic acid
  MISC_FEATURE (24)..(24): Xaa is (S)-2-amino-2-methylhept-6-enoic acid
  MISC_FEATURE (29)..(29): amino acid has C terminal amide
HXQGTFTSDXSKYLDERAAXDFVXWLLDT

SEQ ID NO: 13 - protein, 30 aa, Artificial Sequence
  Peptide
  MISC_FEATURE (21)..(28): Miscellaneous feature: the alkene chain of the amino acid at position 21 forms a double bond containing ring with the alkene chain of the amino acid at position 28
  MISC_FEATURE (2)..(2): Xaa is alpha aminoisobutyric acid
  MISC_FEATURE (10)..(10): Xaa is Lysine conjugated to gamma-Glu-gamma-Glu- C16 fatty acid
  MISC_FEATURE (16)..(16): Xaa is alpha aminoisobutyric acid
  MISC_FEATURE (21)..(21): Xaa is (R)-2-amino-2-methyloct-7-enoic acid
  MISC_FEATURE (28)..(28): Xaa is (S)-2-amino-2-methylnon-8-enoic acid
  MISC_FEATURE (30)..(30): Xaa is C terminal amide
  MISC_FEATURE (30)..(30): Xaa is Lysine conjugated to gamma-Glutamic acid
HXQGTFTSDXSKYLDXRAAQXFVQWLMXTX

SEQ ID NO: 14 - protein, 30 aa, Artificial Sequence
  Peptide
  MISC_FEATURE (24)..(28): Miscellaneous feature: the alkene chain of the amino acid at position 24 forms a double bond containing ring with the alkene chain of the amino acid at position 28
  MISC_FEATURE (2)..(2): Xaa is alpha aminoisobutyric acid
  MISC_FEATURE (10)..(10): Xaa is Lysine conjugated to gamma-Glu-gamma-Glu- C16 fatty acid
  MISC_FEATURE (16)..(16): Xaa is alpha aminoisobutyric acid
  MISC_FEATURE (24)..(24): Xaa is (S)-2-amino-2-methylhept-6-enoic acid
  MISC_FEATURE (28)..(28): Xaa is (S)-2-amino-2-methylhept-6-enoic acid
  MISC_FEATURE (30)..(30): Xaa is C terminal amide
  MISC_FEATURE (30)..(30): Xaa is Lysine conjugated to gamma-Glutamic acid
HXQGTFTSDXSKYLDXRAAQDFVXWLMXTX

SEQ ID NO: 15 - protein, 29 aa, Artificial Sequence
  Peptide
  MISC_FEATURE (20)..(24): Miscellaneous feature: the alkene chain of the amino acid at position 20 forms a double bond containing ring with the alkene chain of the amino acid at position 24
  MISC_FEATURE (2)..(2): Xaa is D-Serine
  MISC_FEATURE (10)..(10): Xaa is Lys conjugated to gamma-Glu-gamma-Glu- C16 fatty acid
  MISC_FEATURE (20)..(20): Xaa is (S)-2-aminohept-6-enoic acid
  MISC_FEATURE (24)..(24): Xaa is (S)-2-aminohept-6-enoic acid
  MISC_FEATURE (29)..(29): amino acid has C terminal amide
HXQGTFTSDXSKYLDERAAXDFVXWLLDT

SEQ ID NO: 16 - protein, 30 aa, Artificial Sequence
  Peptide
  MISC_FEATURE (24)..(28): Miscellaneous feature :the alkene chain of the amino acid at position 24 forms a double bond containing ring with the alkene chain of the amino acid at position 28
  MISC_FEATURE (2)..(2): Xaa is alpha aminoisobutyric acid
  MISC_FEATURE (10)..(10): Xaa is Lysine conjugated to gamma-Glu-gamma-Glu- C16 fatty acid
  MISC_FEATURE (16)..(16): Xaa is alpha aminoisobutyric acid
  MISC_FEATURE (24)..(24): Xaa is (S)-2-aminohept-6-enoic acid
  MISC_FEATURE (28)..(28): Xaa is (S)-2-aminohept-6-enoic acid
  MISC_FEATURE (30)..(30): Xaa is C terminal amide
  MISC_FEATURE (30)..(30): Xaa is Lysine conjugated to gamma-Glutamic acid
HXQGTFTSDXSKYLDXRAAQDFVXWLLXTX

SEQ ID NO: 17 - protein, 29 aa, Artificial Sequence
  Peptide
  MISC_FEATURE (20)..(24): Miscellaneous feature: the alkene chain of the amino acid at position 20 forms a double bond containing ring with the alkene chain of the amino acid at position 24
  MISC_FEATURE (2)..(2): Xaa is D-Serine
  MISC_FEATURE (20)..(20): Xaa is (S)-2-aminohept-6-enoic acid
  MISC_FEATURE (24)..(24): Xaa is (S)-2-aminohept-6-enoic acid
  MISC_FEATURE (29)..(29): amino acid has C terminal amide
HXQGTFTSDKSKYLDERAAXDFVXWLLDT

SEQ ID NO: 18 - protein, 30 aa, Artificial Sequence
  Peptide
  MISC_FEATURE (24)..(28): Miscellaneous feature: the alkene chain of the amino acid at position 24 forms a double bond containing ring with the alkene chain of the amino acid at position 28
  MISC_FEATURE (2)..(2): Xaa is alpha aminoisobutyric acid
  MISC_FEATURE (16)..(16): Xaa is alpha aminoisobutyric acid
  MISC_FEATURE (24)..(24): Xaa is (S)-2-aminohept-6-enoic acid
  MISC_FEATURE (28)..(28): Xaa is (S)-2-aminohept-6-enoic acid
  MISC_FEATURE (30)..(30): Xaa is C terminal amide
  MISC_FEATURE (30)..(30): Xaa is Lysine conjugated to gamma-Glutamic acid
HXQGTFTSDKSKYLDXRAAQDFVXWLLXTX

SEQ ID NO: 19 - protein, 29 aa, Artificial Sequence
  Peptide
  MISC_FEATURE (20)..(24): Miscellaneous feature: the alkene chain of the amino acid at position 20 forms a double bond containing ring with the alkene chain of the amino acid at position 24
  MISC_FEATURE (2)..(2): Xaa is D-Serine
  MISC_FEATURE (20)..(20): Xaa is (S)-2-amino-2-methylhept-6-enoic acid
  MISC_FEATURE (24)..(24): Xaa is (S)-2-amino-2-methylhept-6-enoic acid
  MISC_FEATURE (29)..(29): amino acid has  C terminal amide
HXQGTFTSDKSKYLDERAAXDFVXWLLDT

SEQ ID NO: 20 - protein, 30 aa, Artificial Sequence
  Peptide
  MISC_FEATURE (1)..(30): Miscellaneous feature:  wherein the alkene chain of (R)-2-amino-2-methyloct-7-enoic acid forms a double bond containing ring with the alkene chain of (S)-2-amino-2-methylnon-8-enoic acid; or the alkene chains of
  MISC_FEATURE (2)..(2): Xaa is alpha-aminoisobutyric acid or D-Serine
  MISC_FEATURE (10)..(10): Xaa is Lysine, Lysine conjugated to a fatty acid, or Lysine conjugated to a fatty diacid
  MISC_FEATURE (12)..(12): Xaa is (R)-2-amino-2-methyloct-7-enoic acid, or Lysine
  MISC_FEATURE (16)..(16): Xaa is  alpha-aminoisobutyric acid, or Glutamic acid
  MISC_FEATURE (17)..(17): Xaa is (R)-2-amino-2-methyloct-7-enoic acid, or Arginine
  MISC_FEATURE (19)..(19): Xaa is (S)-2-amino-2-methylnon-8-enoic acid, or Alanine
  MISC_FEATURE (20)..(20): Xaa is Glutamine, (R)-2-amino-2-methyloct-7-enoic acid, (S)-2-amino-2-methylhept-6-enoic acid, or (S)-2-aminohept-6-enoic acid
  MISC_FEATURE (21)..(21): Xaa is Aspartic acid or (R)-2-amino-2-methyloct-7-enoic acid
  MISC_FEATURE (24)..(24): Xaa is  Glutamine, (S)-2-amino-2-methylnon-8-enoic acid, (S)-2-amino-2-methylhept-6-enoic acid, or (S)-2-aminohept-6-enoic acid
  MISC_FEATURE (27)..(27): Xaa is Leucine, (S)-2-amino-2-methylnon-8-enoic acid, or Methionine
  MISC_FEATURE (28)..(28): Xaa is Aspartic acid, (S)-2-amino-2-methylnon-8-enoic acid, (S)-2-amino-2-methylhept-6-enoic acid, or (S)-2-aminohept-6-enoic acid
  MISC_FEATURE (30)..(30): Xaa is absent, or Lysine conjugated by a gamma-glutamic acid spacer
HXQGTFTSDXSXYLDXXAXXXFVXWLXXTX